European Patent Specification EP 3 775 277 B1, published December 3, 2025. Title: Method for diagnosing diseases using multiplex fluorescence and sequencing. Applicant: MultiplexDX. The sequence listing filed with the application follows.

SEQUENCE LISTING (16 sequences)

SEQ ID NO: 1 - DNA, 20 bp, Mus musculus
ggaaaagaaactaaccagga

SEQ ID NO: 2 - DNA, 17 bp, Mus musculus
atcagaccccagaaaag

SEQ ID NO: 3 - DNA, 20 bp, Mus musculus
ctaaggagtgtgtaacaact

SEQ ID NO: 4 - DNA, 19 bp, Mus musculus
ctgaaaatggatggcgctg

SEQ ID NO: 5 - DNA, 15 bp, Mus musculus
cggaacgggacggga

SEQ ID NO: 6 - DNA, 18 bp, Mus musculus
agtcggtcctgagagatg

SEQ ID NO: 7 - DNA, 16 bp, Mus musculus
ggagcagaagggcaaa

SEQ ID NO: 8 - DNA, 17 bp, Mus musculus
tcagtacgagaggaacc

SEQ ID NO: 9 - DNA, 20 bp, artificial
  probe containing LNA
  misc_RNA (3)..(3): LNA residue
  misc_RNA (7)..(7): LNA residue
  misc_RNA (10)..(10): LNA residue
  misc_RNA (13)..(13): LNA residue
  misc_RNA (16)..(16): LNA residue
tcctggttagtttcttttcc

SEQ ID NO: 10 - DNA, 17 bp, artificial
  probe containing LNA
  misc_RNA (2)..(4): LNA residue
  misc_RNA (7)..(7): LNA residue
  misc_RNA (9)..(10): LNA residue
  misc_RNA (13)..(13): LNA residue
  misc_RNA (16)..(16): LNA residue
cttttctggggtctgat

SEQ ID NO: 11 - DNA, 20 bp, artificial
  probe containing LNA
  misc_RNA (4)..(4): LNA residue
  misc_RNA (7)..(7): LNA residue
  misc_RNA (13)..(13): LNA residue
  misc_RNA (16)..(16): LNA residue
  misc_RNA (18)..(19): LNA residue
agttgttacacactccttag

SEQ ID NO: 12 - DNA, 19 bp, artificial
  probe containing LNA
  misc_RNA (4)..(4): LNA residue
  misc_RNA (7)..(7): LNA residue
  misc_RNA (10)..(10): LNA residue
  misc_RNA (13)..(13): LNA residue
  misc_RNA (16)..(16): LNA residue
cagcgccatccattttcag

SEQ ID NO: 13 - DNA, 15 bp, artificial
  probe containing LNA
  misc_RNA (4)..(4): LNA residue
  misc_RNA (7)..(7): LNA residue
  misc_RNA (10)..(10): LNA residue
tcccgtcccgttccg

SEQ ID NO: 14 - DNA, 18 bp, artificial
  probe containing LNA
  misc_RNA (6)..(6): LNA residue
  misc_RNA (8)..(8): LNA residue
  misc_RNA (13)..(13): LNA residue
  misc_RNA (15)..(15): LNA residue
  misc_RNA (17)..(17): LNA residue
catctctcaggaccgact

SEQ ID NO: 15 - DNA, 16 bp, artificial
  probe containing LNA
  misc_RNA (2)..(2): LNA residue
  misc_RNA (7)..(7): LNA residue
  misc_RNA (14)..(14): LNA residue
  misc_RNA (16)..(16): LNA residue
tttgcccttctgctcc

SEQ ID NO: 16 - DNA, 17 bp, artificial
  probe containing LNA
  misc_RNA (4)..(4): LNA residue
  misc_RNA (6)..(6): LNA residue
  misc_RNA (7)..(7): LNA residue
  misc_RNA (9)..(9): LNA residue
  misc_RNA (12)..(12): LNA residue
  misc_RNA (16)..(16): LNA residue
ggttcctctcgtactga